European Patent Application EP 4 242 309 A1, published September 13, 2023. Title: Chimeric Antigen Receptor. Applicant: NATIONAL UNIVERSITY CORPORATION TOKAI NATIONAL HIGHER EDUCATION AND RESEARCH SYSTEM. The sequence listing filed with the application follows.

SEQUENCE LISTING (28 sequences)

SEQ ID NO: 1 - protein, 267 aa, Artificial Sequence
  19CARscFv
MLLLVTSLLLCELPHPAFLLIPDIQMTQTTSSLSASLGDRVTISCRASQDISKYLNWYQQKPDGTVKLLIYHTSRLHSGVPSRFSGSGSGTDYSLTISNLEQEDIATYFCQQGNTLPYTFGGGTKLEITGSTSGSGKPGSGEGSTKGEVKLQESGPGLVAPSQSLSVTCTVSGVSLPDYGVSWIRQPPRKGLEWLGVIWGSETTYYNSALKSRLTIIKDNSKSQVFLKMNSLQTDDTAIYYCAKHYYYGGSYAMDYWGQGTSVTVSS

SEQ ID NO: 2 - protein, 12 aa, Artificial Sequence
  IgG4-Fc
ESKYGPPCPPCP

SEQ ID NO: 3 - protein, 28 aa, Artificial Sequence
  CD28TM
MFWVLVVVGGVLACYSLLVTVAFIIFWV

SEQ ID NO: 4 - protein, 61 aa, Artificial Sequence
  79A
RKRWQNEKLGLDAGDEYEDENLYEGLNLDDCSMYEDISRGLQGTYQDVGSLNIGDVQLEKP

SEQ ID NO: 5 - protein, 62 aa, Artificial Sequence
  CD40
KKVAKKPTNKAPHPKQEPQEINFPDDLPGSNTAAPVQETLHGCQPVTQEDGKESRISVQERQ

SEQ ID NO: 6 - protein, 112 aa, Artificial Sequence
  3z
RVKFSRSADAPAYQQGQNQLYNELNLGRREEYDVLDKRRGRDPEMGGKPRRKNPQEGLYNELQKDKMAEAYSEIGMKGERRRGKGHDGLYQGLSTATKDTYDALHMQALPPR

SEQ ID NO: 7 - protein, 24 aa, Artificial Sequence
  T2A
LEGGGEGRGSLLTCGDVEENPGPR

SEQ ID NO: 8 - protein, 357 aa, Artificial Sequence
  tEGFR
MLLLVTSLLLCELPHPAFLLIPRKVCNGIGIGEFKDSLSINATNIKHFKNCTSISGDLHILPVAFRGDSFTHTPPLDPQELDILKTVKEITGFLLIQAWPENRTDLHAFENLEIIRGRTKQHGQFSLAVVSLNITSLGLRSLKEISDGDVIISGNKNLCYANTINWKKLFGTSGQKTKIISNRGENSCKATGQVCHALCSPEGCWGPEPRDCVSCRNVSRGRECVDKCNLLEGEPREFVENSECIQCHPECLPQAMNITCTGRGPDNCIQCAHYIDGPHCVKTCPAGVMGENNTLVWKYADAGHVCHLCHPNCTYGCTGPGLEGCPTNGPKIPSIATGMVGALLLLLVVALGIGLFM

SEQ ID NO: 9 - protein, 926 aa, Artificial Sequence
  CD79a.40z.SH
MLLLVTSLLLCELPHPAFLLIPDIQMTQTTSSLSASLGDRVTISCRASQDISKYLNWYQQKPDGTVKLLIYHTSRLHSGVPSRFSGSGSGTDYSLTISNLEQEDIATYFCQQGNTLPYTFGGGTKLEITGSTSGSGKPGSGEGSTKGEVKLQESGPGLVAPSQSLSVTCTVSGVSLPDYGVSWIRQPPRKGLEWLGVIWGSETTYYNSALKSRLTIIKDNSKSQVFLKMNSLQTDDTAIYYCAKHYYYGGSYAMDYWGQGTSVTVSSESKYGPPCPPCPMFWVLVVVGGVLACYSLLVTVAFIIFWVRKRWQNEKLGLDAGDEYEDENLYEGLNLDDCSMYEDISRGLQGTYQDVGSLNIGDVQLEKPGGGKKVAKKPTNKAPHPKQEPQEINFPDDLPGSNTAAPVQETLHGCQPVTQEDGKESRISVQERQRVKFSRSADAPAYQQGQNQLYNELNLGRREEYDVLDKRRGRDPEMGGKPRRKNPQEGLYNELQKDKMAEAYSEIGMKGERRRGKGHDGLYQGLSTATKDTYDALHMQALPPRLEGGGEGRGSLLTCGDVEENPGPRMLLLVTSLLLCELPHPAFLLIPRKVCNGIGIGEFKDSLSINATNIKHFKNCTSISGDLHILPVAFRGDSFTHTPPLDPQELDILKTVKEITGFLLIQAWPENRTDLHAFENLEIIRGRTKQHGQFSLAVVSLNITSLGLRSLKEISDGDVIISGNKNLCYANTINWKKLFGTSGQKTKIISNRGENSCKATGQVCHALCSPEGCWGPEPRDCVSCRNVSRGRECVDKCNLLEGEPREFVENSECIQCHPECLPQAMNITCTGRGPDNCIQCAHYIDGPHCVKTCPAGVMGENNTLVWKYADAGHVCHLCHPNCTYGCTGPGLEGCPTNGPKIPSIATGMVGALLLLLVVALGIGLFM

SEQ ID NO: 10 - DNA, 801 bp, Artificial Sequence
  19CARscFv
atgctgctgctggtgaccagcctgctgctgtgcgagctgccccaccccgcctttctgctgatccccgacatccagatgacccagaccacctccagcctgagcgccagcctgggcgaccgggtgaccatcagctgccgggccagccaggacatcagcaagtacctgaactggtatcagcagaagcccgacggcaccgtcaagctgctgatctaccacaccagccggctgcacagcggcgtgcccagccggtttagcggcagcggctccggcaccgactacagcctgaccatctccaacctggaacaggaagatatcgccacctacttttgccagcagggcaacacactgccctacacctttggcggcggaacaaagctggaaatcaccggcagcacctccggcagcggcaagcctggcagcggcgagggcagcaccaagggcgaggtgaagctgcaggaaagcggccctggcctggtggcccccagccagagcctgagcgtgacctgcaccgtgagcggcgtgagcctgcccgactacggcgtgagctggatccggcagccccccaggaagggcctggaatggctgggcgtgatctggggcagcgagaccacctactacaacagcgccctgaagagccggctgaccatcatcaaggacaacagcaagagccaggtgttcctgaagatgaacagcctgcagaccgacgacaccgccatctactactgcgccaagcactactactacggcggcagctacgccatggactactggggccagggcaccagcgtgaccgtgagcagc

SEQ ID NO: 11 - DNA, 36 bp, Artificial Sequence
  IgG4-Fc
gaatctaagtacggaccgccctgccccccttgccct

SEQ ID NO: 12 - DNA, 84 bp, Artificial Sequence
  CD28TM
atgttctgggtgctggtggtggtcggaggcgtgctggcctgctacagcctgctggtcaccgtggccttcatcatcttttgggtg

SEQ ID NO: 13 - DNA, 183 bp, Artificial Sequence
  79A
aggaaacgatggcagaacgagaagctcgggttggatgccggggatgaatatgaagatgaaaacctttatgaaggcctgaacctggacgactgctccatgtatgaggacatctcccggggcctccagggcacctaccaggatgtgggcagcctcaacataggagatgtccagctggagaagccg

SEQ ID NO: 14 - DNA, 186 bp, Artificial Sequence
  CD40
aaaaaggtggccaagaagccaaccaataaggccccccaccccaagcaggaaccccaggagatcaattttcccgacgatcttcctggctccaacactgctgctccagtgcaggagactttacatggatgccaaccggtcacccaggaggatggcaaagagagtcgcatctcagtgcaggagagacag

SEQ ID NO: 15 - DNA, 336 bp, Artificial Sequence
  3z
cgggtgaagttcagcagaagcgccgacgcccctgcctaccagcagggccagaatcagctgtacaacgagctgaacctgggcagaagggaagagtacgacgtcctggataagcggagaggccgggaccctgagatgggcggcaagcctcggcggaagaacccccaggaaggcctgtataacgaactgcagaaagacaagatggccgaggcctacagcgagatcggcatgaagggcgagcggaggcggggcaagggccacgacggcctgtatcagggcctgtccaccgccaccaaggatacctacgacgccctgcacatgcaggccctgcccccaagg

SEQ ID NO: 16 - DNA, 72 bp, Artificial Sequence
  T2A
ctcgagggcggcggagagggcagaggaagtcttctaacatgcggtgacgtggaggagaatcccggccctagg

SEQ ID NO: 17 - DNA, 1074 bp, Artificial Sequence
  tEGFR
atgcttctcctggtgacaagccttctgctctgtgagttaccacacccagcattcctcctgatcccacgcaaagtgtgtaacggaataggtattggtgaatttaaagactcactctccataaatgctacgaatattaaacacttcaaaaactgcacctccatcagtggcgatctccacatcctgccggtggcatttaggggtgactccttcacacatactcctcctctggatccacaggaactggatattctgaaaaccgtaaaggaaatcacagggtttttgctgattcaggcttggcctgaaaacaggacggacctccatgcctttgagaacctagaaatcatacgcggcaggaccaagcaacatggtcagttttctcttgcagtcgtcagcctgaacataacatccttgggattacgctccctcaaggagataagtgatggagatgtgataatttcaggaaacaaaaatttgtgctatgcaaatacaataaactggaaaaaactgtttgggacctccggtcagaaaaccaaaattataagcaacagaggtgaaaacagctgcaaggccacaggccaggtctgccatgccttgtgctcccccgagggctgctggggcccggagcccagggactgcgtctcttgccggaatgtcagccgaggcagggaatgcgtggacaagtgcaaccttctggagggtgagccaagggagtttgtggagaactctgagtgcatacagtgccacccagagtgcctgcctcaggccatgaacatcacctgcacaggacggggaccagacaactgtatccagtgtgcccactacattgacggcccccactgcgtcaagacctgcccggcaggagtcatgggagaaaacaacaccctggtctggaagtacgcagacgccggccatgtgtgccacctgtgccatccaaactgcacctacggatgcactgggccaggtcttgaaggctgtccaacgaatgggcctaagatcccgtccatcgccactgggatggtgggggccctcctcttgctgctggtggtggccctggggatcggcctcttcatgtga

SEQ ID NO: 18 - DNA, 2781 bp, Artificial Sequence
  CD79a.40z.SH
atgctgctgctggtgaccagcctgctgctgtgcgagctgccccaccccgcctttctgctgatccccgacatccagatgacccagaccacctccagcctgagcgccagcctgggcgaccgggtgaccatcagctgccgggccagccaggacatcagcaagtacctgaactggtatcagcagaagcccgacggcaccgtcaagctgctgatctaccacaccagccggctgcacagcggcgtgcccagccggtttagcggcagcggctccggcaccgactacagcctgaccatctccaacctggaacaggaagatatcgccacctacttttgccagcagggcaacacactgccctacacctttggcggcggaacaaagctggaaatcaccggcagcacctccggcagcggcaagcctggcagcggcgagggcagcaccaagggcgaggtgaagctgcaggaaagcggccctggcctggtggcccccagccagagcctgagcgtgacctgcaccgtgagcggcgtgagcctgcccgactacggcgtgagctggatccggcagccccccaggaagggcctggaatggctgggcgtgatctggggcagcgagaccacctactacaacagcgccctgaagagccggctgaccatcatcaaggacaacagcaagagccaggtgttcctgaagatgaacagcctgcagaccgacgacaccgccatctactactgcgccaagcactactactacggcggcagctacgccatggactactggggccagggcaccagcgtgaccgtgagcagcgaatctaagtacggaccgccctgccccccttgccctatgttctgggtgctggtggtggtcggaggcgtgctggcctgctacagcctgctggtcaccgtggccttcatcatcttttgggtgaggaaacgatggcagaacgagaagctcgggttggatgccggggatgaatatgaagatgaaaacctttatgaaggcctgaacctggacgactgctccatgtatgaggacatctcccggggcctccagggcacctaccaggatgtgggcagcctcaacataggagatgtccagctggagaagccgggcggagggaaaaaggtggccaagaagccaaccaataaggccccccaccccaagcaggaaccccaggagatcaattttcccgacgatcttcctggctccaacactgctgctccagtgcaggagactttacatggatgccaaccggtcacccaggaggatggcaaagagagtcgcatctcagtgcaggagagacagcgggtgaagttcagcagaagcgccgacgcccctgcctaccagcagggccagaatcagctgtacaacgagctgaacctgggcagaagggaagagtacgacgtcctggataagcggagaggccgggaccctgagatgggcggcaagcctcggcggaagaacccccaggaaggcctgtataacgaactgcagaaagacaagatggccgaggcctacagcgagatcggcatgaagggcgagcggaggcggggcaagggccacgacggcctgtatcagggcctgtccaccgccaccaaggatacctacgacgccctgcacatgcaggccctgcccccaaggctcgagggcggcggagagggcagaggaagtcttctaacatgcggtgacgtggaggagaatcccggccctaggatgcttctcctggtgacaagccttctgctctgtgagttaccacacccagcattcctcctgatcccacgcaaagtgtgtaacggaataggtattggtgaatttaaagactcactctccataaatgctacgaatattaaacacttcaaaaactgcacctccatcagtggcgatctccacatcctgccggtggcatttaggggtgactccttcacacatactcctcctctggatccacaggaactggatattctgaaaaccgtaaaggaaatcacagggtttttgctgattcaggcttggcctgaaaacaggacggacctccatgcctttgagaacctagaaatcatacgcggcaggaccaagcaacatggtcagttttctcttgcagtcgtcagcctgaacataacatccttgggattacgctccctcaaggagataagtgatggagatgtgataatttcaggaaacaaaaatttgtgctatgcaaatacaataaactggaaaaaactgtttgggacctccggtcagaaaaccaaaattataagcaacagaggtgaaaacagctgcaaggccacaggccaggtctgccatgccttgtgctcccccgagggctgctggggcccggagcccagggactgcgtctcttgccggaatgtcagccgaggcagggaatgcgtggacaagtgcaaccttctggagggtgagccaagggagtttgtggagaactctgagtgcatacagtgccacccagagtgcctgcctcaggccatgaacatcacctgcacaggacggggaccagacaactgtatccagtgtgcccactacattgacggcccccactgcgtcaagacctgcccggcaggagtcatgggagaaaacaacaccctggtctggaagtacgcagacgccggccatgtgtgccacctgtgccatccaaactgcacctacggatgcactgggccaggtcttgaaggctgtccaacgaatgggcctaagatcccgtccatcgccactgggatggtgggggccctcctcttgctgctggtggtggccctggggatcggcctcttcatgtga

SEQ ID NO: 19 - protein, 41 aa, Artificial Sequence
  CD28
RSKRSRLLHSDYMNMTPRRPGPTRKHYQPYARDFAAYRSPP

SEQ ID NO: 20 - DNA, 123 bp, Artificial Sequence
  CD28
aggagtaagaggagcaggctcctgcacagtgactacatgaacatgactccccgccgccccgggcccacccgcaagcattaccagccctatgccccaccacgcgacttcgcagcctatcgctcc

SEQ ID NO: 21 - protein, 42 aa, Artificial Sequence
  4-1BB
KRGRKKLLYIFKQPFMRPVQTTQEEDGCSCRFPEEEEGGCEL

SEQ ID NO: 22 - DNA, 126 bp, Artificial Sequence
  4-1BB
aaacggggcagaaagaaactcctgtatatattcaaacaaccatttatgagaccagtacaaactactcaagaggaagatggctgtagctgccgatttccagaagaagaagaaggaggatgtgaactg

SEQ ID NO: 23 - protein, 232 aa, Artificial Sequence
  LH
EPKSSDKTHTSPPCPAPEFLGGPSVFLFPPKPKDTLMISRTPEVTCVVVDVSQEDPEVQFNWYVDGVEVHNAKTKPREEQFNSTYRVVSVLTVLHQDWLNGKEYKCKVSNKGLPSSIEKTISKAKGQPREPQVYTLPPSQEEMTKNQVSLTCLVKGFYPSDIAVEWESNGQPENNYKTTPPVLDSDGSFFLYSRLTVDKSRWQEGNVFSCSVMHEALHNHYTQKSLSLSLGK

SEQ ID NO: 24 - DNA, 696 bp, Artificial Sequence
  LH
gagcccaaatcttctgacaaaactcacacatctccaccgtgcccagcccccgagttcctgggcggacccagcgtgttcctgttcccccccaagcccaaggacaccctgatgatcagccggacccccgaggtgacctgcgtggtggtggacgtgagccaggaagatcccgaggtccagttcaattggtacgtggacggcgtggaagtgcacaacgccaagaccaagcccagagaggaacagttcaacagcacctaccgggtggtgtctgtgctgaccgtgctgcaccaggactggctgaacggcaaagaatacaagtgcaaggtgtccaacaagggcctgcccagcagcatcgaaaagaccatcagcaaggccaagggccagcctcgcgagccccaggtgtacaccctgcctccctcccaggaagagatgaccaagaaccaggtgtccctgacctgcctggtgaagggcttctaccccagcgacatcgccgtggagtgggagagcaacggccagcctgagaacaactacaagaccacccctcccgtgctggacagcgacggcagcttcttcctgtacagccggctgaccgtggacaagagccggtggcaggaaggcaacgtctttagctgcagcgtgatgcacgaggccctgcacaaccactacacccagaagagcctgagcctgtccctgggcaag

SEQ ID NO: 25 - protein, 243 aa, Artificial Sequence
  37CARscFv
EIVLTQSPATLSLSPGERATLSCRASENVYSYLAWYQQKPGQAPRLLIYFAKTLAEGIPARFSGSGSGTDFTLTISSLEPEDFAVYYCQHHSDNPWTFGQGTKVEIKGSTSGSGKPGSGEGSTKGEVQLVQSGAEVKKPGESLKISCKGSGYSFTGYNMNWVRQMPGKGLEWMGNIDPYYGGTTYNRKFKGQVTISADKSISTAYLQWSSLKASDTAMYYCARSVGPFDSWGQGTLVTVSSDQ

SEQ ID NO: 26 - DNA, 729 bp, Artificial Sequence
  37CARscFv
gaaattgtgttgacacagtctccagccaccctgtctttgtctccaggcgaaagagccaccctctcctgccgagcaagtgaaaatgtttacagctacttagcctggtaccaacagaaacctggccaggctcctaggctcctcatctattttgcaaaaaccttagcagaaggaattccagccaggttcagtggcagtggctccgggacagacttcactctcaccatcagcagcctagagcctgaagattttgcagtttattactgtcaacatcattccgataatccgtggacattcggccaagggaccaaggtggaaatcaaaggcagcacctccggcagcggcaagcctggcagcggcgagggcagcaccaagggcgaggtgcagctggtgcagtctggagcagaggtgaaaaagcccggagagtctctgaagatttcctgtaagggctccggttactcattcactggctacaatatgaactgggtgcgccagatgcccgggaaaggcctcgagtggatgggcaatattgatccttattatggtggtactacctacaaccggaagttcaagggccaggtcactatctccgccgacaagtccatcagcaccgcctacctgcaatggagcagcctgaaggcctcggacaccgccatgtattactgtgcacgctcagtcggccctttcgactcctggggccagggcaccctggtcactgtctcctctgatcag

SEQ ID NO: 27 - protein, 246 aa, Artificial Sequence
  20CARscFv
MTQSPSFLSASVGDRVTITCKASQSVSNDVAWYQQKPGQSPKVLIYFASNRYTGVPDRFSGSGYGTDFTLTISSLQAEDVAVYFCQQDYSSPLTFGAGTKLEIKGGSSRSSSSGGGGSGGGGQIQLVQSGSELKKPGASVKVSCKASGYTFTNFGVNWVRQAPGKGLEWMGWINTYTGEPSYAQGFTGRFVFSLDASVSTAYLQISSLKAEDTATYFCTRRTNYYGTSYYYAMDYWGQGTTVTVSS

SEQ ID NO: 28 - DNA, 738 bp, Artificial Sequence
  20CARscFv
atgacccagagccccagcttcctgagcgccagcgtgggcgaccgcgtgaccatcacctgcaaggccagccagagcgtgagcaacgacgtggcctggtaccagcagaagcccggccagagccccaaggtgctgatctacttcgccagcaaccgctacaccggcgtgcccgaccgcttcagcggcagcggctacggcaccgacttcaccctgaccatcagcagcctgcaggccgaggacgtggccgtgtacttctgccagcaggactacagcagccccctgaccttcggcgccggcaccaagctggagatcaagggcggcagcagccgcagcagcagcagcggcggcggcggcagcggcggcggcggccagatccagctggtgcagagcggcagcgagctgaagaagcccggcgccagcgtgaaggtgagctgcaaggccagcggctacaccttcaccaacttcggcgtgaactgggtgcgccaggcccccggcaagggcctggagtggatgggctggatcaacacctacaccggcgagcccagctacgcccagggcttcaccggccgcttcgtgttcagcctggacgccagcgtgagcaccgcctacctgcagatcagcagcctgaaggccgaggacaccgccacctacttctgcacccgccgcaccaactactacggcaccagctactactacgccatggactactggggccagggcaccaccgtgaccgtctcgagc